European Patent Application EP 4 343 002 A1, published March 27, 2024. Title: COMPOSITION AND METHOD FOR ANALYZING TARGET MOLECULE FROM SAMPLE. Applicant: 10K Genomics. The sequence listing filed with the application follows.

SEQUENCE LISTING (10 sequences)

SEQ ID NO: 1 - DNA, 15 bp, Artificial Sequence
  Primer 1
atccacgtgcttgag

SEQ ID NO: 2 - DNA, 22 bp, Artificial Sequence
  Primer 2
gtggtatcaacgcagagtgatc

SEQ ID NO: 3 - DNA, 17 bp, Artificial Sequence
  Primer 3
cttccgatctggtctcg

SEQ ID NO: 4 - DNA, 22 bp, Artificial Sequence
  Primer 4
cagacgtgtgctcttccgatct

SEQ ID NO: 5 - DNA, 33 bp, Artificial Sequence
  PCR adapter
acactctttccctacacgacgctcttccgatct

SEQ ID NO: 6 - DNA, 15 bp, Artificial Sequence
  Linker 1
cgactcactacaggg

SEQ ID NO: 7 - DNA, 15 bp, Artificial Sequence
  Linker 2
tcggtgacacgatcg

SEQ ID NO: 8 - DNA, 12 bp, Artificial Sequence
  complementary sequence
gctctggctgtc

SEQ ID NO: 9 - DNA, 22 bp, Artificial Sequence
  Probe
agatcggaagagcacacgtctg

SEQ ID NO: 10 - DNA, 22 bp, Artificial Sequence
  Downstream sequence
gatcactctgcgttgataccac